European Patent Application EP 4 137 517 A1, published February 22, 2023. Title: ANTIBODY TO HUMAN INTERLEUKIN-4 RECEPTOR Α, PREPARATION METHOD THEREFOR AND USE THEREOF. Applicant: Shanghai Mabgeek Biotech Co., Ltd. The sequence listing filed with the application follows.

SEQUENCE LISTING (206 sequences)

SEQ ID NO: 1 - DNA, 366 bp, Mus musculus
gaagtgcagctggtggaaagcggcggcggcctggtgaaaccgggcggcagcctgaaactgagctgcgcggcgagcggctttacctttagcgattatggcatgcattgggtgcgccaggcgccggaaaaaggcctggaatgggtggcgtatattaacagcggcagcagcaaaatttatcatgcggataccgtgaaaggccgctttaccattagccgcgataacgcgaaaaacaccctgtttctgcagatgaccagcctgcgcagcgaagataccgcgatgtattattgcgcgcgctttccgaccgtggtggcggcgcgctatccgatggattattggggccagggcaccagcgtgaccgtgagcagc

SEQ ID NO: 2 - protein, 122 aa, Mus musculus
EVQLVESGGGLVKPGGSLKLSCAASGFTFSDYGMHWVRQAPEKGLEWVAYINSGSSKIYHADTVKGRFTISRDNAKNTLFLQMTSLRSEDTAMYYCARFPTVVAARYPMDYWGQGTSVTVSS

SEQ ID NO: 3 - DNA, 321 bp, Mus musculus
gatattcagatgacccagaccccgagcagcctgagcgcgagcctgggcgatcgcgtgaccattagctgccgcgcgagccaggatattagcaactatctgaactggtatcagcagaaaccggatggcaccgtgaaactgctgatttattttaccagccgcctgcatagcggcgtgccgagccgctttagcggcggcggcagcggcaccgattatagcctgaccattagcaacctggaacaggaagatattgcgacctatttttgccagcagggcaacaccctgccgtatacctttggcggcggcaccaaactggaaattaaa

SEQ ID NO: 4 - protein, 107 aa, Mus musculus
DIQMTQTPSSLSASLGDRVTISCRASQDISNYLNWYQQKPDGTVKLLIYFTSRLHSGVPSRFSGGGSGTDYSLTISNLEQEDIATYFCQQGNTLPYTFGGGTKLEIK

SEQ ID NO: 5 - DNA, 354 bp, Mus musculus
gaagtgcagctggtggaaagcggcggcggcctggtgaaaccgggcggcagcctgaaactgagctgcgcggcgagcggctttacctttagcgattatggcattcattgggtgcgccaggcgccggataaaggcctggaatgggtggcgtatattcgcagcgatagcagcattattcattatgcggataccgtgaaaggccgctttaccattagccgcgataacgcgaaaaacaccctgtttctgcagatgaccagcctgcgcagcgaagataccgcgatgtattattgcacccgcggccgcgatcgcggctattttgattattggggccagggcaccaccctgaccgtgagcagc

SEQ ID NO: 6 - protein, 118 aa, Mus musculus
EVQLVESGGGLVKPGGSLKLSCAASGFTFSDYGIHWVRQAPDKGLEWVAYIRSDSSIIHYADTVKGRFTISRDNAKNTLFLQMTSLRSEDTAMYYCTRGRDRGYFDYWGQGTTLTVSS

SEQ ID NO: 7 - DNA, 318 bp, Mus musculus
cagattgtgctgacccagagcccggcgctgatgagcgcgagcccgggcgaaaaagtgaccatgacctgcagcgcgagcagcagcgtgagctatatgtattggtatcagcagaaaccgcgcagcagcccgaaaccgtggatttatctgaccagcaacctggcgagcggcgtgccggcgcgctttagcggcagcggcagcggcaccagctatagcctgaccattagcagcatggaagcggaagatgcggcgacctattattgccagcagtggaccagcattccgtttacctttggcagcggcaccaaactggaaattaaa

SEQ ID NO: 8 - protein, 106 aa, Mus musculus
QIVLTQSPALMSASPGEKVTMTCSASSSVSYMYWYQQKPRSSPKPWIYLTSNLASGVPARFSGSGSGTSYSLTISSMEAEDAATYYCQQWTSIPFTFGSGTKLEIK

SEQ ID NO: 9 - DNA, 366 bp, Mus musculus
gaagtgcagctggtggaaagcggcggcggcctggtgaaaccgggcggcagcctgaaactgagctgcgcggcgagcggctttacctttagcgattatggcatgcattgggtgcgccaggcgccggaaaaaggcctggaatgggtggcgtatattagcagcggcagcaccaccatttattatgcggataccgtgaaaggccgctttaccattagccgcgataacggcaaaaacaccctgtttctgcagatgaccagcctgcgcagcgaagataccgcgatgtattattgcgcgcgcattagcaccgtggtggcgaaacgctatgcgatggattattggggccagggcaccagcgtgaccgtgagcagc

SEQ ID NO: 10 - protein, 122 aa, Mus musculus
EVQLVESGGGLVKPGGSLKLSCAASGFTFSDYGMHWVRQAPEKGLEWVAYISSGSTTIYYADTVKGRFTISRDNGKNTLFLQMTSLRSEDTAMYYCARISTVVAKRYAMDYWGQGTSVTVSS

SEQ ID NO: 11 - DNA, 321 bp, Mus musculus
gatattcagatgacccagaccgcgagcagcctgagcgcgagcctgggcgatcgcgtgaccattagctgccgcgcgagccaggatattagcaactatctgaactggtatcagcagaaaccggatggcaccgtgaaactgctgatttattataccagccgcctgcatagcggcgtgccgagccgctttagcggcagcggcagcggcaccgattatagcctgaccattagcaacctggaacaggaagatattgcgacctatttttgccagcagattaacgcgctgccgctgacctttggcgcgggcaccaaactggaactgaaa

SEQ ID NO: 12 - protein, 107 aa, Mus musculus
DIQMTQTASSLSASLGDRVTISCRASQDISNYLNWYQQKPDGTVKLLIYYTSRLHSGVPSRFSGSGSGTDYSLTISNLEQEDIATYFCQQINALPLTFGAGTKLELK

SEQ ID NO: 13 - DNA, 366 bp, Mus musculus
gaagtgcagctggtggaaagcggcggcggcctggtgaaaccgggcggcagcctgaaactgagctgcgcggcgagcggctttacctttagcgattatggcatgcattgggtgcgccaggcgccggaaaaaggcctggaatgggtggcgtatattagcagcggcagcagcaccatttattatgcggataccgtgaaaggccgctttaccattagccgcgataacgcgaaaaacaccctgtttctgcagatgaccagcctgcgcagcgaagataccgcgatgtattattgcgcgcgcattagcaccgtggtggcgaaacgctatgcgatggattattggggccagggcaccagcgtgaccgtgagcagc

SEQ ID NO: 14 - protein, 122 aa, Mus musculus
EVQLVESGGGLVKPGGSLKLSCAASGFTFSDYGMHWVRQAPEKGLEWVAYISSGSSTIYYADTVKGRFTISRDNAKNTLFLQMTSLRSEDTAMYYCARISTVVAKRYAMDYWGQGTSVTVSS

SEQ ID NO: 15 - DNA, 321 bp, Mus musculus
gatattcagatgacccagaccgcgagcagcctgagcgcgagcctgggcgatcgcgtgaccattagctgccgcgcgagccaggatattagcaactatctgaactggtatcagcagaaaccggatggcaccgtgaaactgctgatttattataccagccgcctgcatagcggcgtgccgagccgctttagcggcagcggcagcggcaccgattatagcctgaccattagcaacctggaacaggaagatattgcgacctatttttgccaggaagtgaacatgctgccgctgacctttggcgcgggcaccaaactggaactgaaa

SEQ ID NO: 16 - protein, 107 aa, Mus musculus
DIQMTQTASSLSASLGDRVTISCRASQDISNYLNWYQQKPDGTVKLLIYYTSRLHSGVPSRFSGSGSGTDYSLTISNLEQEDIATYFCQEVNMLPLTFGAGTKLELK

SEQ ID NO: 17 - DNA, 366 bp, Mus musculus; identical to SEQ ID NO: 9

SEQ ID NO: 18 - protein, 122 aa, Mus musculus; identical to SEQ ID NO: 10

SEQ ID NO: 19 - DNA, 321 bp, Mus musculus; identical to SEQ ID NO: 11

SEQ ID NO: 20 - protein, 107 aa, Mus musculus; identical to SEQ ID NO: 12

SEQ ID NO: 21 - DNA, 360 bp, Mus musculus
gaagtgcagctgcagcagagcggcccggaactggtgaaaccgggcgcgagcgtgaaaattccgtgcaaagcgagcggctatacctttaccgattataacatggattgggtgaaacagagccatggcaaaagcctggaatggattggcgatattaacccgaacaacggcaacattctgtttaaccagaaatttaaaggcaaagcgaccctgaccgtggataaaagcagcagcaccgcgtatgtggaactgcgcagcctgaccagcgaagataccgcggtgtattattgcggccgcggcggcctgcgccgccgcggctttatggattattggggccagggcaccagcgtgaccgtgagcagc

SEQ ID NO: 22 - protein, 120 aa, Mus musculus
EVQLQQSGPELVKPGASVKIPCKASGYTFTDYNMDWVKQSHGKSLEWIGDINPNNGNILFNQKFKGKATLTVDKSSSTAYVELRSLTSEDTAVYYCGRGGLRRRGFMDYWGQGTSVTVSS

SEQ ID NO: 23 - DNA, 318 bp, Mus musculus
cagattgtgctgagccagagcccggcgattctgagcgcgagcccgggcgaaaaagtgaccatgacctgccgcgcgagcagcagcgtgagctatatgcattggtatcagcagaaaccgggcagcagcccgaaaccgtggatttatgcggcgagcaacctggcgagcggcgtgccggcgcgctttagcggcagcggcagcggcaccagctatagcctgaccattagccgcgtggaagcggaagatgcggcgacctattattgccagcagtggagcagcaacccgccgacctttggcggcggcaccaaactggaaattaaa

SEQ ID NO: 24 - protein, 106 aa, Mus musculus
QIVLSQSPAILSASPGEKVTMTCRASSSVSYMHWYQQKPGSSPKPWIYAASNLASGVPARFSGSGSGTSYSLTISRVEAEDAATYYCQQWSSNPPTFGGGTKLEIK

SEQ ID NO: 25 - DNA, 360 bp, Mus musculus
gatgtgcagctgcagcagagcggcccggaactgctgaaaccgggcgcgagcgtgaaaattccgtgccaggcgagcggctatacctttaccgattataacatggattgggtgaaacagagccatggcaaaaacctggaatggattggcaacattaacccgaacaacggcggcaccttttataaccagaaatttaaaggcaaagcgaccctgaccgtggataaaagcagcagcaccgcgtatatggaactgcgcagcctgaccagcgaagataccgcggtgtattattgcggccgcggcggcctgcgccgccgcggctttatggattattggggccagggcaccagcgtgaccgtgagcagc

SEQ ID NO: 26 - protein, 120 aa, Mus musculus
DVQLQQSGPELLKPGASVKIPCQASGYTFTDYNMDWVKQSHGKNLEWIGNINPNNGGTFYNQKFKGKATLTVDKSSSTAYMELRSLTSEDTAVYYCGRGGLRRRGFMDYWGQGTSVTVSS

SEQ ID NO: 27 - DNA, 318 bp, Mus musculus
cagattgtgctgagccagagcccggcgattctgagcgcgagcccgggcgaaaaagtgaccatgacctgccgcgcgagcagcagcgtgatttatattcattggtatcagcagaaaccgggcagcagcccgaaaccgtggatttatgcggcgagcaacctggcgagcggcgtgccggtgcgctttagcggcagcggcagcggcaccagctatagcctgaccattagccgcgtggaagcggaagatgcggcgacctattattgccagcagtggagcgtgaacccgccgacctttggcggcggcaccaaactggaaattaaa

SEQ ID NO: 28 - protein, 106 aa, Mus musculus
QIVLSQSPAILSASPGEKVTMTCRASSSVIYIHWYQQKPGSSPKPWIYAASNLASGVPVRFSGSGSGTSYSLTISRVEAEDAATYYCQQWSVNPPTFGGGTKLEIK

SEQ ID NO: 29 - DNA, 360 bp, Mus musculus; identical to SEQ ID NO: 21

SEQ ID NO: 30 - protein, 120 aa, Mus musculus; identical to SEQ ID NO: 22

SEQ ID NO: 31 - DNA, 318 bp, Mus musculus; identical to SEQ ID NO: 23

SEQ ID NO: 32 - protein, 106 aa, Mus musculus; identical to SEQ ID NO: 24

SEQ ID NO: 33 - DNA, 360 bp, Mus musculus
gaagtgcagctgcagcagagcggcccggaactggtgaaaccgggcgcgagcgtgaaaattagctgcaaagcgagcggctatacctttaccgattataacatggattgggtgaaacagagccatggcaaaagcctggaatggattggcaccaccaacccgaacaacggcggcaccctgtataaccagaaatttaaaggcaaagcgaccctgaccgtggataaaagcagcagcaccgcgtatatggaactgcgcagcctgaccagcgaagataccgcggtgtattattgcgcgcgcggcggcctgcgccgccgcggctttgtggattattggggccagggcaccagcgtgaccgtgagcagc

SEQ ID NO: 34 - protein, 120 aa, Mus musculus
EVQLQQSGPELVKPGASVKISCKASGYTFTDYNMDWVKQSHGKSLEWIGTTNPNNGGTLYNQKFKGKATLTVDKSSSTAYMELRSLTSEDTAVYYCARGGLRRRGFVDYWGQGTSVTVSS

SEQ ID NO: 35 - DNA, 318 bp, Mus musculus
cagattgtgctgagccagagcccggcgattctgagcgcgagcccgggcgaaaaagtgaccatgacctgccgcgcgagcagcagcgtgaactatctgcattggtatcagcagaaaccgggcagcagcccgaaaccgtggatttatgcgaccagcaacctggcgagcggcgtgccggcgcgctttagcggcagcggcagcggcaccagctatagcctgaccattagccgcgtggaagcggaagatgcggcgacctattattgccagcagtggagcagcaacccgccgacctttggcggcggcaccaaactggaaattaaa

SEQ ID NO: 36 - protein, 106 aa, Mus musculus
QIVLSQSPAILSASPGEKVTMTCRASSSVNYLHWYQQKPGSSPKPWIYATSNLASGVPARFSGSGSGTSYSLTISRVEAEDAATYYCQQWSSNPPTFGGGTKLEIK

SEQ ID NO: 37 - DNA, 360 bp, Mus musculus; identical to SEQ ID NO: 21

SEQ ID NO: 38 - protein, 120 aa, Mus musculus; identical to SEQ ID NO: 22

SEQ ID NO: 39 - DNA, 318 bp, Mus musculus; identical to SEQ ID NO: 23

SEQ ID NO: 40 - protein, 106 aa, Mus musculus; identical to SEQ ID NO: 24

SEQ ID NO: 41 - DNA, 360 bp, Mus musculus; identical to SEQ ID NO: 25

SEQ ID NO: 42 - protein, 120 aa, Mus musculus; identical to SEQ ID NO: 26

SEQ ID NO: 43 - DNA, 318 bp, Mus musculus
cagattgtgctgagccagagcccggcgattctgagcgcgagcccgggcgaaaaagtgaccatgacctgccgcgcgagcagcagcgtgatttatattcattggtatcagcagaaaccgggcagcagcccgaaaccgtggatttatgcggcgagcaacctggcgagcggcgtgccggcgcgctttagcggcagcggcagcggcaccagctatagcctgaccattagccgcgtggaagcggaagatgcggcgacctattattgccagcagtggagcgtgaacccgccgacctttggcggcggcaccaaactggaaattaaa

SEQ ID NO: 44 - protein, 106 aa, Mus musculus
QIVLSQSPAILSASPGEKVTMTCRASSSVIYIHWYQQKPGSSPKPWIYAASNLASGVPARFSGSGSGTSYSLTISRVEAEDAATYYCQQWSVNPPTFGGGTKLEIK

SEQ ID NO: 45 - DNA, 360 bp, Mus musculus
gaagtgcagctgcagcagagcggcccggaactggtgaaaccgggcgcgagcgtgaaaattccgtgcaaagcgagcggctatacctttaccgattataacatggattgggtgaaacagagccgcggcaaaagcctggaatggattggcaccattaacccgaacaacggcgataccatgtataaccagaaatttaaagataaagcgaccctgaccgtggataaaagcagcaccaccgcgtatatggaactgcgcagcctgaccagcgaagataccgcggtgtattattgcggccgcggcggcctgcgccgccgcggctttatggattattggggccgcggcaccagcgtgaccgtgagcagc

SEQ ID NO: 46 - protein, 120 aa, Mus musculus
EVQLQQSGPELVKPGASVKIPCKASGYTFTDYNMDWVKQSRGKSLEWIGTINPNNGDTMYNQKFKDKATLTVDKSSTTAYMELRSLTSEDTAVYYCGRGGLRRRGFMDYWGRGTSVTVSS

SEQ ID NO: 47 - DNA, 318 bp, Mus musculus
cagattgtgctgagccagagcccggcgattctgagcgcgagcccgggcgaaaaagtgaccatgacctgccgcgcgagcagcagcgtgatttatattcattggtatcagcagaaaccgggcagcagcccgaaaccgtggatttatgcgattagcaacctggcgagcggcgtgccggcgcgctttagcggcagcggcagcggcaccagctattttctgaccattagccgcgtggaagtggaagatgcggcgacctattattgccagcagtggagcgtgaacccgccgacctttggcggcggcaccaaactggaaattaaa

SEQ ID NO: 48 - protein, 106 aa, Mus musculus
QIVLSQSPAILSASPGEKVTMTCRASSSVIYIHWYQQKPGSSPKPWIYAISNLASGVPARFSGSGSGTSYFLTISRVEVEDAATYYCQQWSVNPPTFGGGTKLEIK

SEQ ID NO: 49 - DNA, 360 bp, Mus musculus
gatgtgcagctgcagcagagcggccgcgaactgctgaaacgcggcgcgagcgtgaaaattccgtgccaggcgagcggctatacctttaccgattataacatggattgggtgaaacagagccatggcaaaaacctggaatggattggcaacattaacccgaacaacggcggcaccttttataaccagaaatttaaaggcaaagcgaccctgaccgtggataaaagcagcagcaccgcgtatatggaactgcgcagcctgaccagcgaagataccgcggtgtattattgcggccgcggcggcctgcgccgccgcggctttatggattattggggccagggcaccagcgtgaccgtgagcagc

SEQ ID NO: 50 - protein, 120 aa, Mus musculus
DVQLQQSGRELLKRGASVKIPCQASGYTFTDYNMDWVKQSHGKNLEWIGNINPNNGGTFYNQKFKGKATLTVDKSSSTAYMELRSLTSEDTAVYYCGRGGLRRRGFMDYWGQGTSVTVSS

SEQ ID NO: 51 - DNA, 318 bp, Mus musculus; identical to SEQ ID NO: 43

SEQ ID NO: 52 - protein, 106 aa, Mus musculus; identical to SEQ ID NO: 44

SEQ ID NO: 53 - DNA, 360 bp, Mus musculus
gatgtgcagctgcagcagagcggcccggaactgctgaaaccgggcgcgagcgtgaaaattccgtgccaggcgagcggctatacctttaccgattataacatggattgggtgaaacagagccatggcaaaaacctggaatggattggcaccattaacccgaacaacggcggcaccttttataaccagaactttaaaggcaaagcgaccctgaccgtggataaaagcagcagcaccgcgtgcatggaactgcgcagcctgaccagcgatgataccgcggtgtattattgcggccgcggcggcctgcgccgccgcggctttatggattattggggccagggcaccagcgtgaccgtgagcagc

SEQ ID NO: 54 - protein, 120 aa, Mus musculus
DVQLQQSGPELLKPGASVKIPCQASGYTFTDYNMDWVKQSHGKNLEWIGTINPNNGGTFYNQNFKGKATLTVDKSSSTACMELRSLTSDDTAVYYCGRGGLRRRGFMDYWGQGTSVTVSS

SEQ ID NO: 55 - DNA, 318 bp, Mus musculus; identical to SEQ ID NO: 43

SEQ ID NO: 56 - protein, 106 aa, Mus musculus; identical to SEQ ID NO: 44

SEQ ID NO: 57 - DNA, 360 bp, Mus musculus
gatgtgcagctgcagcagagcggcccggaactgctgaaaccgggcgcgagcgtgaaaattccgtgccaggcgagcggctatacctttaccgattataacatggattgggtgaaacagagccatggcaaaaacctggaatggattggcaacattaacccgaacaacggcggcaccttttataaccagaaatttaaaggcaaagcgaccctgaccgtggataaaagcagcagcaccgcgtatatggaactgcgcagcctgaccagcgaagataccgcggtgtattattgcggccgcggcggcctgcgccgccgcggctttctggattattggggccagggcaccagcgtgaccgtgagcagc

SEQ ID NO: 58 - protein, 120 aa, Mus musculus
DVQLQQSGPELLKPGASVKIPCQASGYTFTDYNMDWVKQSHGKNLEWIGNINPNNGGTFYNQKFKGKATLTVDKSSSTAYMELRSLTSEDTAVYYCGRGGLRRRGFLDYWGQGTSVTVSS

SEQ ID NO: 59 - DNA, 318 bp, Mus musculus
cagattgtgctgagccagagcccggcgattctgagcgcgagcccgggcgaaaaagtgaccatgacctgccgcgcgagcagcagcgtgatttatattcattggtatcagcagaaaccgggcagcagcccgaaaccgtggatttatgcggtgagcaacctggcgagcggcgtgccggtgcgctttagcggcagcggcagcggcaccagctatagcctgaccattagccgcgtggaagcggaagatgcggcgacctattattgccagcagtggagcgtgaacccgccgacctttggcggcggcaccaaactggaaattaaa

SEQ ID NO: 60 - protein, 106 aa, Mus musculus
QIVLSQSPAILSASPGEKVTMTCRASSSVIYIHWYQQKPGSSPKPWIYAVSNLASGVPVRFSGSGSGTSYSLTISRVEAEDAATYYCQQWSVNPPTFGGGTKLEIK

SEQ ID NO: 61 - DNA, 360 bp, Mus musculus; identical to SEQ ID NO: 25

SEQ ID NO: 62 - protein, 120 aa, Mus musculus; identical to SEQ ID NO: 26

SEQ ID NO: 63 - DNA, 318 bp, Mus musculus; identical to SEQ ID NO: 43

SEQ ID NO: 64 - protein, 106 aa, Mus musculus; identical to SEQ ID NO: 44

SEQ ID NO: 65 - DNA, 360 bp, Mus musculus
gaagtgcagctgcagcagagcggcccggaactggtgaaaccgggcgcgagcgtgaaaattccgtgcaaagcgagcggctatacctttaccgattataacgtggattgggtgaaacagagccatggccagagcctggattggattggcaccattaacccgaacaacggcggcattctgagcaaccagaaatttaaaggcaaagcgaccctgaccgtggataccagcagcagcaccgcgtatatggaactgcgcagcctgaccagcgaagataccgcggtgtattattgcggccgcggcggcctgcgccgccgcggctttatggattattggggccagggcaccagcgtgaccgtgagcagc

SEQ ID NO: 66 - protein, 120 aa, Mus musculus
EVQLQQSGPELVKPGASVKIPCKASGYTFTDYNVDWVKQSHGQSLDWIGTINPNNGGILSNQKFKGKATLTVDTSSSTAYMELRSLTSEDTAVYYCGRGGLRRRGFMDYWGQGTSVTVSS

SEQ ID NO: 67 - DNA, 318 bp, Mus musculus
cagattgtgctgagccagagcccggcgattctgagcgcgagcccgggcgaaaaagtgaccatgacctgccgcgcgagcagcagcgtgatttatattcattggtattatcagaaagcgggcagcagcccgaaaccgtggatttatgcggcgagcaacctgccgagcggcgtgccggcgcgctttagcggcagcggcagcggcaccagctatagcctgaccattagccgcgtggaagcggaagatgcggcgacctattattgccagcagtggagcagcaacccgccgacctttggcggcggcaccaaactggaaattaaa

SEQ ID NO: 68 - protein, 106 aa, Mus musculus
QIVLSQSPAILSASPGEKVTMTCRASSSVIYIHWYYQKAGSSPKPWIYAASNLPSGVPARFSGSGSGTSYSLTISRVEAEDAATYYCQQWSSNPPTFGGGTKLEIK

SEQ ID NO: 69 - DNA, 366 bp, Synthetic
gaagtgcagctggtggaaagcggcggcggcctggtgcagccgggcggcagcctgcgcctgagctgcgcggcgagcggctttacctttagcgattatggcatgcattgggtgcgccaggcgccgggcaaaggcctggaatgggtggcgtatattaacagcggcagcagcaaaatttatcatgcggataccgtgaaaggccgctttaccattagccgcgataacgcgaaaaacagcctgtatctgcagatgaacagcctgcgcgcggaagataccgcggtgtattattgcgcgcgctttccgaccgtggtggcggcgcgctatccgatggattattggggccagggcaccctggtgaccgtgagcagc

SEQ ID NO: 70 - protein, 122 aa, Synthetic
EVQLVESGGGLVQPGGSLRLSCAASGFTFSDYGMHWVRQAPGKGLEWVAYINSGSSKIYHADTVKGRFTISRDNAKNSLYLQMNSLRAEDTAVYYCARFPTVVAARYPMDYWGQGTLVTVSS

SEQ ID NO: 71 - protein, 448 aa, Synthetic
EVQLVESGGGLVQPGGSLRLSCAASGFTFSDYGMHWVRQAPGKGLEWVAYINSGSSKIYHADTVKGRFTISRDNAKNSLYLQMNSLRAEDTAVYYCARFPTVVAARYPMDYWGQGTLVTVSSASTKGPSVFPLAPCSRSTSESTAALGCLVKDYFPEPVTVSWNSGALTSGVHTFPAVLQSSGLYSLSSVVTVPSSSLGTKTYTCNVDHKPSNTKVDKRVESKYGPPCPPCPAPEFLGGPSVFLFPPKPKDTLMISRTPEVTCVVVDVSQEDPEVQFNWYVDGVEVHNAKTKPREEQFNSTYRVVSVLTVLHQDWLNGKEYKCKVSNKGLPSSIEKTISKAKGQPREPQVYTLPPSQEEMTKNQVSLTCLVKGFYPSDIAVEWESNGQPENNYKTTPPVLDSDGSFFLYSRLTVDKSRWQEGNVFSCSVMHEALHNHYTQKSLSLSLG

SEQ ID NO: 72 - DNA, 321 bp, Synthetic
gatattcagatgacccagagcccgagcagcctgagcgcgagcgtgggcgatcgcgtgaccattacctgccgcgcgagccaggatattagcaactatctgaactggtatcagcagaaaccgggcaaagcgccgaaactgctgatttattttaccagccgcctgcatagcggcgtgccgagccgctttagcggcagcggcagcggcaccgattataccctgaccattagcagcctgcagccggaagattttgcgacctattattgccagcagggcaacaccctgccgtatacctttggccagggcaccaaactggaaattaaa

SEQ ID NO: 73 - protein, 107 aa, Synthetic
DIQMTQSPSSLSASVGDRVTITCRASQDISNYLNWYQQKPGKAPKLLIYFTSRLHSGVPSRFSGSGSGTDYTLTISSLQPEDFATYYCQQGNTLPYTFGQGTKLEIK

SEQ ID NO: 74 - protein, 214 aa, Synthetic
DIQMTQSPSSLSASVGDRVTITCRASQDISNYLNWYQQKPGKAPKLLIYFTSRLHSGVPSRFSGSGSGTDYTLTISSLQPEDFATYYCQQGNTLPYTFGQGTKLEIKRTVAAPSVFIFPPSDEQLKSGTASVVCLLNNFYPREAKVQWKVDNALQSGNSQESVTEQDSKDSTYSLSSTLTLSKADYEKHKVYACEVTHQGLSSPVTKSFNRGEC

SEQ ID NO: 75 - DNA, 354 bp, Synthetic
gaagtgcagctggtggaaagcggcggcggcctggtgcagccgggcggcagcctgcgcctgagctgcgcggcgagcggctttacctttagcgattatggcattcattgggtgcgccaggcgccgggcaaaggcctggaatgggtgagctatattcgcagcgatagcagcattattcattatgcggataccgtgaaaggccgctttaccattagccgcgataacgcgaaaaacagcctgtatctgcagatgaacagcctgcgcgcggaagataccgcggtgtattattgcgcgcgcggccgcgatcgcggctattttgattattggggccagggcaccctggtgaccgtgagcagc

SEQ ID NO: 76 - protein, 118 aa, Synthetic
EVQLVESGGGLVQPGGSLRLSCAASGFTFSDYGIHWVRQAPGKGLEWVSYIRSDSSIIHYADTVKGRFTISRDNAKNSLYLQMNSLRAEDTAVYYCARGRDRGYFDYWGQGTLVTVSS

SEQ ID NO: 77 - protein, 444 aa, Synthetic
EVQLVESGGGLVQPGGSLRLSCAASGFTFSDYGIHWVRQAPGKGLEWVSYIRSDSSIIHYADTVKGRFTISRDNAKNSLYLQMNSLRAEDTAVYYCARGRDRGYFDYWGQGTLVTVSSASTKGPSVFPLAPCSRSTSESTAALGCLVKDYFPEPVTVSWNSGALTSGVHTFPAVLQSSGLYSLSSVVTVPSSSLGTKTYTCNVDHKPSNTKVDKRVESKYGPPCPPCPAPEFLGGPSVFLFPPKPKDTLMISRTPEVTCVVVDVSQEDPEVQFNWYVDGVEVHNAKTKPREEQFNSTYRVVSVLTVLHQDWLNGKEYKCKVSNKGLPSSIEKTISKAKGQPREPQVYTLPPSQEEMTKNQVSLTCLVKGFYPSDIAVEWESNGQPENNYKTTPPVLDSDGSFFLYSRLTVDKSRWQEGNVFSCSVMHEALHNHYTQKSLSLSLG

SEQ ID NO: 78 - DNA, 318 bp, Synthetic
gaaattgtgctgacccagagcccggcgaccctgagcctgagcccgggcgaacgcgcgaccctgagctgcagcgcgagcagcagcgtgagctatatgtattggtatcagcagaaaccgggccaggcgccgcgcccgtggatttatctgaccagcaacctggcgagcggcgtgccggcgcgctttagcggcagcggcagcggcaccgattttaccctgaccattagcagcctggaaccggaagattttgcggtgtattattgccagcagtggaccagcattccgtttacctttggccagggcaccaaagtggaaattaaa

SEQ ID NO: 79 - protein, 106 aa, Synthetic
EIVLTQSPATLSLSPGERATLSCSASSSVSYMYWYQQKPGQAPRPWIYLTSNLASGVPARFSGSGSGTDFTLTISSLEPEDFAVYYCQQWTSIPFTFGQGTKVEIK

SEQ ID NO: 80 - protein, 213 aa, Synthetic
EIVLTQSPATLSLSPGERATLSCSASSSVSYMYWYQQKPGQAPRPWIYLTSNLASGVPARFSGSGSGTDFTLTISSLEPEDFAVYYCQQWTSIPFTFGQGTKVEIKRTVAAPSVFIFPPSDEQLKSGTASVVCLLNNFYPREAKVQWKVDNALQSGNSQESVTEQDSKDSTYSLSSTLTLSKADYEKHKVYACEVTHQGLSSPVTKSFNRGEC

SEQ ID NO: 81 - DNA, 366 bp, Synthetic
gaagtgcagctggtggaaagcggcggcggcctggtgcagccgggcggcagcctgcgcctgagctgcgcggcgagcggctttacctttagcgattatggcatgcattgggtgcgccaggcgccgggcaaaggcctggaatgggtgagctatattagcagcggcagcagcaccatttattatgcggataccgtgaaaggccgctttaccattagccgcgataacgcgaaaaacagcctgtatctgcagatgaacagcctgcgcgcggaagataccgcggtgtattattgcgcgcgcattagcaccgtggtggcgaaacgctatgcgatggattattggggccagggcaccctggtgaccgtgagcagc

SEQ ID NO: 82 - protein, 122 aa, Synthetic
EVQLVESGGGLVQPGGSLRLSCAASGFTFSDYGMHWVRQAPGKGLEWVSYISSGSSTIYYADTVKGRFTISRDNAKNSLYLQMNSLRAEDTAVYYCARISTVVAKRYAMDYWGQGTLVTVSS

SEQ ID NO: 83 - protein, 448 aa, Synthetic
EVQLVESGGGLVQPGGSLRLSCAASGFTFSDYGMHWVRQAPGKGLEWVSYISSGSSTIYYADTVKGRFTISRDNAKNSLYLQMNSLRAEDTAVYYCARISTVVAKRYAMDYWGQGTLVTVSSASTKGPSVFPLAPCSRSTSESTAALGCLVKDYFPEPVTVSWNSGALTSGVHTFPAVLQSSGLYSLSSVVTVPSSSLGTKTYTCNVDHKPSNTKVDKRVESKYGPPCPPCPAPEFLGGPSVFLFPPKPKDTLMISRTPEVTCVVVDVSQEDPEVQFNWYVDGVEVHNAKTKPREEQFNSTYRVVSVLTVLHQDWLNGKEYKCKVSNKGLPSSIEKTISKAKGQPREPQVYTLPPSQEEMTKNQVSLTCLVKGFYPSDIAVEWESNGQPENNYKTTPPVLDSDGSFFLYSRLTVDKSRWQEGNVFSCSVMHEALHNHYTQKSLSLSLG

SEQ ID NO: 84 - DNA, 321 bp, Synthetic
gatattcagatgacccagagcccgagcagcctgagcgcgagcgtgggcgatcgcgtgaccattacctgccgcgcgagccaggatattagcaactatctgaactggtatcagcagaaaccgggcaaagcgccgaaactgctgatttattataccagccgcctgcatagcggcgtgccgagccgctttagcggcagcggcagcggcaccgattttaccctgaccattagcagcctgcagccggaagatattgcgacctattattgccaggaagtgaacatgctgccgtttacctttggccagggcaccaaagtggaaattaaa

SEQ ID NO: 85 - protein, 107 aa, Synthetic
DIQMTQSPSSLSASVGDRVTITCRASQDISNYLNWYQQKPGKAPKLLIYYTSRLHSGVPSRFSGSGSGTDFTLTISSLQPEDIATYYCQEVNMLPFTFGQGTKVEIK

SEQ ID NO: 86 - protein, 214 aa, Synthetic
DIQMTQSPSSLSASVGDRVTITCRASQDISNYLNWYQQKPGKAPKLLIYYTSRLHSGVPSRFSGSGSGTDFTLTISSLQPEDIATYYCQEVNMLPFTFGQGTKVEIKRTVAAPSVFIFPPSDEQLKSGTASVVCLLNNFYPREAKVQWKVDNALQSGNSQESVTEQDSKDSTYSLSSTLTLSKADYEKHKVYACEVTHQGLSSPVTKSFNRGEC

SEQ ID NO: 87 - DNA, 366 bp, Synthetic
gaagtgcagctggtggaaagcggcggcggcctggtgcagccgggcggcagcctgcgcctgagctgcgcggcgagcggctttacctttagcgattatggcatgcattgggtgcgccaggcgccgggcaaaggcctggaatgggtgagctatattagcagcggcagcaccaccatttattatgcggataccgtgaaaggccgctttaccattagccgcgataacgcgaaaaacagcctgtatctgcagatgaacagcctgcgcgcggaagataccgcggtgtattattgcgcgcgcattagcaccgtggtggcgaaacgctatgcgatggattattggggccagggcaccctggtgaccgtgagcagc

SEQ ID NO: 88 - protein, 122 aa, Synthetic
EVQLVESGGGLVQPGGSLRLSCAASGFTFSDYGMHWVRQAPGKGLEWVSYISSGSTTIYYADTVKGRFTISRDNAKNSLYLQMNSLRAEDTAVYYCARISTVVAKRYAMDYWGQGTLVTVSS

SEQ ID NO: 89 - protein, 448 aa, Synthetic
EVQLVESGGGLVQPGGSLRLSCAASGFTFSDYGMHWVRQAPGKGLEWVSYISSGSTTIYYADTVKGRFTISRDNAKNSLYLQMNSLRAEDTAVYYCARISTVVAKRYAMDYWGQGTLVTVSSASTKGPSVFPLAPCSRSTSESTAALGCLVKDYFPEPVTVSWNSGALTSGVHTFPAVLQSSGLYSLSSVVTVPSSSLGTKTYTCNVDHKPSNTKVDKRVESKYGPPCPPCPAPEFLGGPSVFLFPPKPKDTLMISRTPEVTCVVVDVSQEDPEVQFNWYVDGVEVHNAKTKPREEQFNSTYRVVSVLTVLHQDWLNGKEYKCKVSNKGLPSSIEKTISKAKGQPREPQVYTLPPSQEEMTKNQVSLTCLVKGFYPSDIAVEWESNGQPENNYKTTPPVLDSDGSFFLYSRLTVDKSRWQEGNVFSCSVLHEALHSHYTQKSLSLSLG

SEQ ID NO: 90 - DNA, 321 bp, Synthetic
gatattcagatgacccagagcccgagcagcctgagcgcgagcgtgggcgatcgcgtgaccattacctgccgcgcgagccaggatattagcaactatctgaactggtatcagcagaaaccgggcaaagcgccgaaactgctgatttattataccagccgcctgcatagcggcgtgccgagccgctttagcggcagcggcagcggcaccgattttaccctgaccattagcagcctgcagccggaagatattgcgacctattattgccagcagattaacgcgctgccgtttacctttggccagggcaccaaactggaaattaaa

SEQ ID NO: 91 - protein, 107 aa, Synthetic
DIQMTQSPSSLSASVGDRVTITCRASQDISNYLNWYQQKPGKAPKLLIYYTSRLHSGVPSRFSGSGSGTDFTLTISSLQPEDIATYYCQQINALPFTFGQGTKLEIK

SEQ ID NO: 92 - protein, 214 aa, Synthetic
DIQMTQSPSSLSASVGDRVTITCRASQDISNYLNWYQQKPGKAPKLLIYYTSRLHSGVPSRFSGSGSGTDFTLTISSLQPEDIATYYCQQINALPFTFGQGTKLEIKRTVAAPSVFIFPPSDEQLKSGTASVVCLLNNFYPREAKVQWKVDNALQSGNSQESVTEQDSKDSTYSLSSTLTLSKADYEKHKVYACEVTHQGLSSPVTKSFNRGEC

SEQ ID NO: 93 - DNA, 360 bp, Synthetic
caggtgcagctggtgcagagcggcgcggaagtgaaaaaaccgggcgcgagcgtgaaagtgagctgcaaagcgagcggctatacctttaccgattataacatggattgggtgcgccaggcgccgggccagaacctggaatggattggcaacattaacccgaacaacggcggcaccttttataaccagaaatttaaaggccgcgcgaccctgaccgtggataaaagcgcgagcaccgcgtatatggaactgagcagcctgcgcagcgaagataccgcggtgtattattgcgcgcgcggcggcctgcgccgccgcggctttatggattattggggccagggcaccctggtgaccgtgagcagc

SEQ ID NO: 94 - protein, 120 aa, Synthetic
QVQLVQSGAEVKKPGASVKVSCKASGYTFTDYNMDWVRQAPGQNLEWIGNINPNNGGTFYNQKFKGRATLTVDKSASTAYMELSSLRSEDTAVYYCARGGLRRRGFMDYWGQGTLVTVSS

SEQ ID NO: 95 - protein, 446 aa, Synthetic
QVQLVQSGAEVKKPGASVKVSCKASGYTFTDYNMDWVRQAPGQNLEWIGNINPNNGGTFYNQKFKGRATLTVDKSASTAYMELSSLRSEDTAVYYCARGGLRRRGFMDYWGQGTLVTVSSASTKGPSVFPLAPCSRSTSESTAALGCLVKDYFPEPVTVSWNSGALTSGVHTFPAVLQSSGLYSLSSVVTVPSSSLGTKTYTCNVDHKPSNTKVDKRVESKYGPPCPPCPAPEFLGGPSVFLFPPKPKDTLMISRTPEVTCVVVDVSQEDPEVQFNWYVDGVEVHNAKTKPREEQFNSTYRVVSVLTVLHQDWLNGKEYKCKVSNKGLPSSIEKTISKAKGQPREPQVYTLPPSQEEMTKNQVSLTCLVKGFYPSDIAVEWESNGQPENNYKTTPPVLDSDGSFFLYSRLTVDKSRWQEGNVFSCSVMHEALHNHYTQKSLSLSLG

SEQ ID NO: 96 - DNA, 318 bp, Synthetic
gaaattgtgctgacccagagcccggcgaccctgagcctgagcccgggcgaacgcgcgaccctgagctgccgcgcgagcagcagcgtgatttatattcattggtatcagcagaaaccgggccagagcccgcgcccgtggatttatgcggcgagcaacctggcgagcggcgtgccggcgcgctttagcggcagcggcagcggcaccgattataccctgaccattagccgcctggaaccggaagattttgcggtgtattattgccagcagtggagcgtgaacccgccgacctttggccagggcaccaaactggaaattaaa

SEQ ID NO: 97 - protein, 106 aa, Synthetic
EIVLTQSPATLSLSPGERATLSCRASSSVIYIHWYQQKPGQSPRPWIYAASNLASGVPARFSGSGSGTDYTLTISRLEPEDFAVYYCQQWSVNPPTFGQGTKLEIK

SEQ ID NO: 98 - protein, 213 aa, Synthetic
EIVLTQSPATLSLSPGERATLSCRASSSVIYIHWYQQKPGQSPRPWIYAASNLASGVPARFSGSGSGTDYTLTISRLEPEDFAVYYCQQWSVNPPTFGQGTKLEIKRTVAAPSVFIFPPSDEQLKSGTASVVCLLNNFYPREAKVQWKVDNALQSGNSQESVTEQDSKDSTYSLSSTLTLSKADYEKHKVYACEVTHQGLSSPVTKSFNRGEC

SEQ ID NO: 99 - DNA, 360 bp, Synthetic
caggtgcagctggtgcagagcggcgcggaagtgaaaaaaccgggcgcgagcgtgaaagtgagctgcaaagcgagcggctatacctttaccgattataacgtggattgggtgcgccaggcgccgggccagggcctggaatggattggcaccattaacccgaacaacggcggcattctgagcaaccagaaatttaaaggccgcgtgaccattaccgtggataccagcgcgagcaccgcgtatatggaactgagcagcctgcgcagcgaagataccgcggtgtattattgcggccgcggcggcctgcgccgccgcggctttatggattattggggccagggcaccctggtgaccgtgagcagc

SEQ ID NO: 100 - protein, 120 aa, Synthetic
QVQLVQSGAEVKKPGASVKVSCKASGYTFTDYNVDWVRQAPGQGLEWIGTINPNNGGILSNQKFKGRVTITVDTSASTAYMELSSLRSEDTAVYYCGRGGLRRRGFMDYWGQGTLVTVSS

SEQ ID NO: 101 - protein, 446 aa, Synthetic
QVQLVQSGAEVKKPGASVKVSCKASGYTFTDYNVDWVRQAPGQGLEWIGTINPNNGGILSNQKFKGRVTITVDTSASTAYMELSSLRSEDTAVYYCGRGGLRRRGFMDYWGQGTLVTVSSASTKGPSVFPLAPCSRSTSESTAALGCLVKDYFPEPVTVSWNSGALTSGVHTFPAVLQSSGLYSLSSVVTVPSSSLGTKTYTCNVDHKPSNTKVDKRVESKYGPPCPPCPAPEFLGGPSVFLFPPKPKDTLMISRTPEVTCVVVDVSQEDPEVQFNWYVDGVEVHNAKTKPREEQFNSTYRVVSVLTVLHQDWLNGKEYKCKVSNKGLPSSIEKTISKAKGQPREPQVYTLPPSQEEMTKNQVSLTCLVKGFYPSDIAVEWESNGQPENNYKTTPPVLDSDGSFFLYSRLTVDKSRWQEGNVFSCSVMHEALHNHYTQKSLSLSLG

SEQ ID NO: 102 - DNA, 318 bp, Synthetic
gaaattgtgctgacccagagcccggcgaccctgagcctgagcccgggcgaacgcgcgaccctgagctgccgcgcgagcagcagcgtgatttatattcattggtatcagcagaaaccgggccaggcgccgcgcccgtggatttatgcggcgagcaacctgccgagcggcgtgccggcgcgctttagcggcagcggcagcggcaccgattttaccctgaccattagcagcctggaaccggaagattttgcggtgtattattgccagcagtggagcagcaacccgccgacctttggccagggcaccaaagtggaaattaaa

SEQ ID NO: 103 - protein, 106 aa, Synthetic
EIVLTQSPATLSLSPGERATLSCRASSSVIYIHWYQQKPGQAPRPWIYAASNLPSGVPARFSGSGSGTDFTLTISSLEPEDFAVYYCQQWSSNPPTFGQGTKVEIK

SEQ ID NO: 104 - protein, 213 aa, Synthetic
EIVLTQSPATLSLSPGERATLSCRASSSVIYIHWYQQKPGQAPRPWIYAASNLPSGVPARFSGSGSGTDFTLTISSLEPEDFAVYYCQQWSSNPPTFGQGTKVEIKRTVAAPSVFIFPPSDEQLKSGTASVVCLLNNFYPREAKVQWKVDNALQSGNSQESVTEQDSKDSTYSLSSTLTLSKADYEKHKVYACEVTHQGLSSPVTKSFNRGEC

SEQ ID NO: 105 - protein, 5 aa, Mus musculus
DYGMH

SEQ ID NO: 106 - protein, 17 aa, Mus musculus
YINSGSSKIYHADTVKG

SEQ ID NO: 107 - protein, 15 aa, Mus musculus
ARFPTVVAARYPMDY

SEQ ID NO: 108 - protein, 11 aa, Mus musculus
RASQDISNYLN

SEQ ID NO: 109 - protein, 7 aa, Mus musculus
FTSRLHS

SEQ ID NO: 110 - protein, 9 aa, Mus musculus
QQGNTLPYT

SEQ ID NO: 111 - protein, 5 aa, Mus musculus
DYGIH

SEQ ID NO: 112 - protein, 17 aa, Mus musculus
YIRSDSSIIHYADTVKG

SEQ ID NO: 113 - protein, 11 aa, Mus musculus
TRGRDRGYFDY

SEQ ID NO: 114 - protein, 10 aa, Mus musculus
SASSSVSYMY

SEQ ID NO: 115 - protein, 7 aa, Mus musculus
LTSNLAS

SEQ ID NO: 116 - protein, 9 aa, Mus musculus
QQWTSIPFT

SEQ ID NO: 117 - protein, 5 aa, Mus musculus
DYGMH

SEQ ID NO: 118 - protein, 17 aa, Mus musculus
YISSGSTTIYYADTVKG

SEQ ID NO: 119 - protein, 15 aa, Mus musculus
ARISTVVAKRYAMDY

SEQ ID NO: 120 - protein, 11 aa, Mus musculus
RASQDISNYLN

SEQ ID NO: 121 - protein, 7 aa, Mus musculus
YTSRLHS

SEQ ID NO: 122 - protein, 9 aa, Mus musculus
QQINALPLT

SEQ ID NO: 123 - protein, 5 aa, Mus musculus
DYGMH

SEQ ID NO: 124 - protein, 17 aa, Mus musculus
YISSGSSTIYYADTVKG

SEQ ID NO: 125 - protein, 15 aa, Mus musculus
ARISTVVAKRYAMDY

SEQ ID NO: 126 - protein, 11 aa, Mus musculus
RASQDISNYLN

SEQ ID NO: 127 - protein, 7 aa, Mus musculus
YTSRLHS

SEQ ID NO: 128 - protein, 9 aa, Mus musculus
QEVNMLPLT

SEQ ID NO: 129 - protein, 5 aa, Mus musculus
DYGMH

SEQ ID NO: 130 - protein, 17 aa, Mus musculus
YISSGSTTIYYADTVKG

SEQ ID NO: 131 - protein, 15 aa, Mus musculus
ARISTVVAKRYAMDY

SEQ ID NO: 132 - protein, 11 aa, Mus musculus
RASQDISNYLN

SEQ ID NO: 133 - protein, 7 aa, Mus musculus
YTSRLHS

SEQ ID NO: 134 - protein, 9 aa, Mus musculus
QQINALPLT

SEQ ID NO: 135 - protein, 5 aa, Mus musculus
DYNMD

SEQ ID NO: 136 - protein, 17 aa, Mus musculus
DINPNNGNILFNQKFKG

SEQ ID NO: 137 - protein, 13 aa, Mus musculus
GRGGLRRRGFMDY

SEQ ID NO: 138 - protein, 10 aa, Mus musculus
RASSSVSYMH

SEQ ID NO: 139 - protein, 7 aa, Mus musculus
AASNLAS

SEQ ID NO: 140 - protein, 9 aa, Mus musculus
QQWSSNPPT

SEQ ID NO: 141 - protein, 5 aa, Mus musculus
DYNMD

SEQ ID NO: 142 - protein, 17 aa, Mus musculus
NINPNNGGTFYNQKFKG

SEQ ID NO: 143 - protein, 13 aa, Mus musculus
GRGGLRRRGFMDY

SEQ ID NO: 144 - protein, 10 aa, Mus musculus
RASSSVIYIH

SEQ ID NO: 145 - protein, 7 aa, Mus musculus
AASNLAS

SEQ ID NO: 146 - protein, 9 aa, Mus musculus
QQWSVNPPT

SEQ ID NO: 147 - protein, 5 aa, Mus musculus
DYNMD

SEQ ID NO: 148 - protein, 17 aa, Mus musculus
DINPNNGNILFNQKFKG

SEQ ID NO: 149 - protein, 13 aa, Mus musculus
GRGGLRRRGFMDY

SEQ ID NO: 150 - protein, 10 aa, Mus musculus
RASSSVSYMH

SEQ ID NO: 151 - protein, 7 aa, Mus musculus
AASNLAS

SEQ ID NO: 152 - protein, 9 aa, Mus musculus
QQWSSNPPT

SEQ ID NO: 153 - protein, 5 aa, Mus musculus
DYNMD

SEQ ID NO: 154 - protein, 17 aa, Mus musculus
TTNPNNGGTLYNQKFKG

SEQ ID NO: 155 - protein, 13 aa, Mus musculus
ARGGLRRRGFVDY

SEQ ID NO: 156 - protein, 10 aa, Mus musculus
RASSSVNYLH

SEQ ID NO: 157 - protein, 7 aa, Mus musculus
ATSNLAS

SEQ ID NO: 158 - protein, 9 aa, Mus musculus
QQWSSNPPT

SEQ ID NO: 159 - protein, 5 aa, Mus musculus
DYNMD

SEQ ID NO: 160 - protein, 17 aa, Mus musculus
DINPNNGNILFNQKFKG

SEQ ID NO: 161 - protein, 13 aa, Mus musculus
GRGGLRRRGFMDY

SEQ ID NO: 162 - protein, 10 aa, Mus musculus
RASSSVSYMH

SEQ ID NO: 163 - protein, 7 aa, Mus musculus
AASNLAS

SEQ ID NO: 164 - protein, 9 aa, Mus musculus
QQWSSNPPT

SEQ ID NO: 165 - protein, 5 aa, Mus musculus
DYNMD

SEQ ID NO: 166 - protein, 17 aa, Mus musculus
NINPNNGGTFYNQKFKG

SEQ ID NO: 167 - protein, 13 aa, Mus musculus
GRGGLRRRGFMDY

SEQ ID NO: 168 - protein, 10 aa, Mus musculus
RASSSVIYIH

SEQ ID NO: 169 - protein, 7 aa, Mus musculus
AASNLAS

SEQ ID NO: 170 - protein, 9 aa, Mus musculus
QQWSVNPPT

SEQ ID NO: 171 - protein, 5 aa, Mus musculus
DYNMD

SEQ ID NO: 172 - protein, 17 aa, Mus musculus
TINPNNGDTMYNQKFKD

SEQ ID NO: 173 - protein, 13 aa, Mus musculus
GRGGLRRRGFMDY

SEQ ID NO: 174 - protein, 10 aa, Mus musculus
RASSSVIYIH

SEQ ID NO: 175 - protein, 7 aa, Mus musculus
AISNLAS

SEQ ID NO: 176 - protein, 9 aa, Mus musculus
QQWSVNPPT

SEQ ID NO: 177 - protein, 5 aa, Mus musculus
DYNMD

SEQ ID NO: 178 - protein, 17 aa, Mus musculus
NINPNNGGTFYNQKFKG

SEQ ID NO: 179 - protein, 13 aa, Mus musculus
GRGGLRRRGFMDY

SEQ ID NO: 180 - protein, 10 aa, Mus musculus
RASSSVIYIH

SEQ ID NO: 181 - protein, 7 aa, Mus musculus
AASNLAS

SEQ ID NO: 182 - protein, 9 aa, Mus musculus
QQWSVNPPT

SEQ ID NO: 183 - protein, 5 aa, Mus musculus
DYNMD

SEQ ID NO: 184 - protein, 17 aa, Mus musculus
TINPNNGGTFYNQNFKG

SEQ ID NO: 185 - protein, 13 aa, Mus musculus
GRGGLRRRGFMDY

SEQ ID NO: 186 - protein, 10 aa, Mus musculus
RASSSVIYIH

SEQ ID NO: 187 - protein, 7 aa, Mus musculus
AASNLAS

SEQ ID NO: 188 - protein, 9 aa, Mus musculus
QQWSVNPPT

SEQ ID NO: 189 - protein, 5 aa, Mus musculus
DYNMD

SEQ ID NO: 190 - protein, 17 aa, Mus musculus
NINPNNGGTFYNQKFKG

SEQ ID NO: 191 - protein, 13 aa, Mus musculus
GRGGLRRRGFLDY

SEQ ID NO: 192 - protein, 10 aa, Mus musculus
RASSSVIYIH

SEQ ID NO: 193 - protein, 7 aa, Mus musculus
AVSNLAS

SEQ ID NO: 194 - protein, 9 aa, Mus musculus
QQWSVNPPT

SEQ ID NO: 195 - protein, 5 aa, Mus musculus
DYNMD

SEQ ID NO: 196 - protein, 17 aa, Mus musculus
NINPNNGGTFYNQKFKG

SEQ ID NO: 197 - protein, 13 aa, Mus musculus
GRGGLRRRGFMDY

SEQ ID NO: 198 - protein, 10 aa, Mus musculus
RASSSVIYIH

SEQ ID NO: 199 - protein, 7 aa, Mus musculus
AASNLAS

SEQ ID NO: 200 - protein, 9 aa, Mus musculus
QQWSVNPPT

SEQ ID NO: 201 - protein, 5 aa, Mus musculus
DYNVD

SEQ ID NO: 202 - protein, 17 aa, Mus musculus
TINPNNGGILSNQKFKG

SEQ ID NO: 203 - protein, 13 aa, Mus musculus
GRGGLRRRGFMDY

SEQ ID NO: 204 - protein, 10 aa, Mus musculus
RASSSVIYIH

SEQ ID NO: 205 - protein, 7 aa, Mus musculus
AASNLPS

SEQ ID NO: 206 - protein, 9 aa, Mus musculus
QQWSSNPPT